European Patent Specification EP 3 322 722 B1, published March 5, 2025. Title: New Monoclonal Anti-Alpha-Synuclein Antibodies. Applicant: H. Lundbeck A/S. The sequence listing filed with the application follows.

SEQUENCE LISTING (43 sequences)

SEQ ID NO: 1 - protein, 10 aa, Artificial
  GM37 CDR 1 Heavy Chain
GFTFSSYAMT

SEQ ID NO: 2 - protein, 17 aa, Artificial
  GM37 CDR2 Heavy Chain
AIRSNGDRTDYADSVKG

SEQ ID NO: 3 - protein, 9 aa, Artificial
  GM37 CDR3 Heavy Chain
AKNWAPFDS

SEQ ID NO: 4 - protein, 11 aa, Artificial
  GM37 CDR1 Light Chain
ASQSVSSSYLA

SEQ ID NO: 5 - protein, 7 aa, Artificial
  GM37 CDR 2 Light Chain
GASSRAT

SEQ ID NO: 6 - protein, 9 aa, Artificial
  GM37 CDR 3 Light Chain
QQYGSSPWT

SEQ ID NO: 7 - protein, 116 aa, Artificial
  GM37 CDR Heavy Chain
EVQLLESGGGLVQTGGSLRLSCAASGFTFSSYAMTWVRQAPGKGLEWVSAIRSNGDRTDYADSVKGRFTISRDNSQNTLYLQMNSLRAEDTAVYYCAKNWAPFDSWGQGTLVTVSS

SEQ ID NO: 8 - protein, 108 aa, Artificial
  GM 37 Light Chain
EIVLTQSPGTLSLSPGERATLSCRASQSVSSSYLAWYQQKPGQAPRLLIYGASSRATGIPDRFSGSGSGTDFTLTISRLEPEDFAVYYCQQYGSSPWTFGQGTKVEIK

SEQ ID NO: 9 - protein, 6 aa, Artificial
  Epitope 112-117
ILEDMP

SEQ ID NO: 10 - protein, 140 aa, Artificial
  Alpha-synuclein
MDVFMKGLSKAKEGVVAAAEKTKQGVAEAAGKTKEGVLYVGSKTKEGVVHGVATVAEKTKEQVTNVGGAVVTGVTAVAQKTVEGAGSIAAATGFVKKDQLGKNEEGAPQEGILEDMPVDPDNEAYEMPSEEGYQDYEPEA

SEQ ID NO: 11 - protein, 165 aa, Artificial
  A-Syn-AAKK-BAP
MDVFMKGLSKAKEGVVAAAEKTKQGVAEAAGKTKEGVLYVGSKTKEGVVHGVATVAEKTKEQVTNVGGAVVTGVTAVAQKTVEGAGNIAAATGLVKKDQLAKQNEEGFLQEGMVNNTDIPVDPENEAYEMPPEEEYQDYEPEAGSAGGSGGLNDIFEAQKIEWHE

SEQ ID NO: 12 - protein, 165 aa, Artificial
  A-Syn-BAAK-BAP
MDVFMKGLSMAKEGVVAAAEKTKQGVTEAAEKTKEGVLYVGSKTKEGVVHGVATVAEKTKEQVTNVGGAVVTGVTAVAQKTVEGAGSIAAATGFVKKDQLAKQNEEGFLQEGMVNNTDIPVDPENEAYEMPPEEEYQDYEPEAGSAGGSGGLNDIFEAQKIEWHE

SEQ ID NO: 13 - protein, 162 aa, Artificial
  A-Syn-BBAA-BAP
MDVFMKGLSMAKEGVVAAAEKTKQGVTEAAEKTKEGVLYVGSKTREGVVQGVASVAEKTKEQASHLGGAVVTGVTAVAQKTVEGAGSIAAATGFVKKDQLGKNEEGAPQEGILEDMPVDPDNEAYEMPSEEGYQDYEPEAGSAGGSGGLNDIFEAQKIEWHE

SEQ ID NO: 14 - protein, 165 aa, Artificial
  A-Syn-BBKK-BAP
MDVFMKGLSMAKEGVVAAAEKTKQGVTEAAEKTKEGVLYVGSKTREGVVQGVASVAEKTKEQASHLGGAVVTGVTAVAQKTVEGAGNIAAATGLVKKDQLAKQNEEGFLQEGMVNNTDIPVDPENEAYEMPPEEEYQDYEPEAGSAGGSGGLNDIFEAQKIEWHE

SEQ ID NO: 15 - protein, 141 aa, Artificial
  A-Syn-120-140_Del-BAP
MDVFMKGLSKAKEGVVAAAEKTKQGVAEAAGKTKEGVLYVGSKTKEGVVHGVATVAEKTKEQVTNVGGAVVTGVTAVAQKTVEGAGSIAAATGFVKKDQLGKNEEGAPQEGILEDMPVDGSAGGSGGLNDIFEAQKIEWHE

SEQ ID NO: 16 - protein, 131 aa, Artificial
  alpha-synuclein amino acids 1-119
MAHHHHHHIEGRMDVFMKGLSKAKEGVVAAAEKTKQGVAEAAGKTKEGVLYVGSKTKEGVVHGVATVAEKTKEQVTNVGGAVVTGVTAVAQKTVEGAGSIAAATGFVKKDQLGKNEEGAPQEGILEDMPVD

SEQ ID NO: 17 - protein, 106 aa, artificial
  kappa (LC constant region)
TVAAPSVFIFPPSDEQLKSGTASVVCLLNNFYPREAKVQWKVDNALQSGNSQESVTEQDSKDSTYSLSSTLTLSKADYEKHKVYACEVTHQGLSSPVTKSFNRGEC

SEQ ID NO: 18 - protein, 329 aa, Artificial
  IgG1 (HC Constant region)
ASTKGPSVFPLAPSSKSTSGGTAALGCLVKDYFPEPVTVSWNSGALTSGVHTFPAVLQSSGLYSLSSVVTVPSSSLGTQTYICNVNHKPSNTKVDKRVEPKSCDKTHTCPPCPAPELLGGPSVFLFPPKPKDTLMISRTPEVTCVVVDVSHEDPEVKFNWYVDGVEVHNAKTKPREEQYNSTYRVVSVLTVLHQDWLNGKEYKCKVSNKALPAPIEKTISKAKGQPREPQVYTLPPSREEMTKNQVSLTCLVKGFYPSDIAVEWESNGQPENNYKTTPPVLDSDGSFFLYSKLTVDKSRWQQGNVFSCSVMHEALHNHYTQKSLSLSPG

SEQ ID NO: 19 - protein, 4 aa, Artificial
  GM285 epitope 112-115
ILED

SEQ ID NO: 20 - protein, 13 aa, Artificial
  GM285 CDR1 Heavy Chain
AASGFTFSRFTMT

SEQ ID NO: 21 - protein, 17 aa, Artificial
  GM285 CDR2 Heavy Chain
AISGSGGGTSYADSVKG

SEQ ID NO: 22 - protein, 9 aa, Artificial
  GM285 CDR3 Heavy Chain
AKNWAPFDY

SEQ ID NO: 23 - protein, 12 aa, Artificial
  GM285 CDR1 Light Chain
RASQSVSRSYLA

SEQ ID NO: 24 - protein, 7 aa, Artificial
  GM285 CDR2 Light Chain
GASSRAT

SEQ ID NO: 25 - protein, 9 aa, Artificial
  GM285 CDR3 Light Chain
QQYGSSPWT

SEQ ID NO: 26 - protein, 116 aa, Artificial
  GM285 VH
EVQLLESGGGLVQPGGSLRLSCAASGFTFSRFTMTWVRQAPGKGLEWVSAISGSGGGTSYADSVKGRLTVSRDNSKNTLYLQMNSLRAEDTAVYYCAKNWAPFDYWGQGTLVTVSS

SEQ ID NO: 27 - protein, 108 aa, Artificial
  GM285 VL
EIVLTQSPGTLSLSPGERATLSCRASQSVSRSYLAWYQQKPGQAPRLLIYGASSRATGIPDRFSGSGSGTDFTLTVSRLEPEDFAVYYCQQYGSSPWTFGQGTKVEIK

SEQ ID NO: 28 - protein, 329 aa, Artificial; identical to SEQ ID NO: 18
  GM285 IgG1 constant region

SEQ ID NO: 29 - protein, 106 aa, Artificial; identical to SEQ ID NO: 17
  GM285 Kappa chain

SEQ ID NO: 30 - protein, 116 aa, Artificial
  GM37 Variant 1 heavy chain
EVQLLESGGGLVQTGGSLRLSCAASGFTFSSYAMTWVRQAPGKGLEWVSAIRSSGDRTDYADSVKGRFTISRDNSQNTLYLQMNSLRAEDTAVYYCAKNWAPFDSWGQGTLVTVSS

SEQ ID NO: 31 - protein, 116 aa, Artificial
  GM 37 variant 2 heavy chain
EVQLLESGGGLVQTGGSLRLSCAASGFTFSSYAMTWVRQAPGKGLEWVSAIRSQGDRTDYADSVKGRFTISRDNSQNTLYLQMNSLRAEDTAVYYCAKNWAPFDSWGQGTLVTVSS

SEQ ID NO: 32 - protein, 116 aa, Artificial
  GM 37 variant 3 heavy chain
EVQLLESGGGLVQTGGSLRLSCAASGFTFSSYAMTWVRQAPGKGLEWVSAIRSHGDRTDYADSVKGRFTISRDNSQNTLYLQMNSLRAEDTAVYYCAKNWAPFDSWGQGTLVTVSS

SEQ ID NO: 33 - protein, 17 aa, Artificial
  GM37 variant 1 heavy chain CDR 2
AIRSSGDRTDYADSVKG

SEQ ID NO: 34 - protein, 17 aa, Artificial
  GM37 variant 2 CDR 2 heavy chain
AIRSQGDRTDYADSVKG

SEQ ID NO: 35 - protein, 17 aa, Artificial
  GM37 variant 3 CDR 2 heavy chain
AIRSHGDRTDYADSVKG

SEQ ID NO: 36 - protein, 5 aa, Artificial
  9E4 binding epitope
NEAYE

SEQ ID NO: 37 - protein, 134 aa, Artificial
  HUMAN Beta-synuclein
MDVFMKGLSMAKEGVVAAAEKTKQGVTEAAEKTKEGVLYVGSKTREGVVQGVASVAEKTKEQASHLGGAVFSGAGNIAAATGLVKREEFPTDLKPEEVAQEAAEEPLIEPLMEPEGESYEDPPQEEYQEYEPEA

SEQ ID NO: 38 - protein, 127 aa, Artificial
  HUMAN Gamma-synuclein
MDVFKKGFSIAKEGVVGAVEKTKQGVTEAAEKTKEGVMYVGAKTKENVVQSVTSVAEKTKEQANAVSEAVVSSVNTVATKTVEEAENIAVTSGVVRKEDLRPSAPQQEGEASKEKEEVAEEAQSGGD

SEQ ID NO: 39 - protein, 140 aa, Artificial
  alpha-synuclein ortholog for Cynomolgus monkey
MDVFMKGLSKAKEGVVAAAEKTKQGVAEAAGKTKEGVLYVGSKTKEGVVHGVATVAEKTKEQVTNVGGAVVTGVTAVAQKTVEGAGSIAAATGFIKKDQLGKNEEGAPQEGILQDMPVDPDNEAYEMPSEEGYQDYEPEA

SEQ ID NO: 40 - protein, 140 aa, Artificial
  alpha-synuclein ortholog for Rat
MDVFMKGLSKAKEGVVAAAEKTKQGVAEAAGKTKEGVLYVGSKTKEGVVHGVTTVAEKTKEQVTNVGGAVVTGVTAVAQKTVEGAGNIAAATGFVKKDQMGKGEEGYPQEGILEDMPVDPSSEAYEMPSEEGYQDYEPEA

SEQ ID NO: 41 - protein, 140 aa, Artificial [sequence omitted]

SEQ ID NO: 42 - protein, 446 aa, artificial
  9E4 HC
EVQLVESGGGLVQPGGSLRLSCAASGFTFSNYGMSWVRQAPGKGLEWVASISSGGGSTYYPDNVKGRFTISRDNAKNSLYLQMNSLRAEDTAVYYCARGGAGIDYWGQGTLVTVSSASTKGPSVFPLAPSSKSTSGGTAALGCLVKDYFPEPVTVSWNSGALTSGVHTFPAVLQSSGLYSLSSVVTVPSSSLGTQTYICNVNHKPSNTKVDKRVEPKSCDKTHTCPPCPAPELLGGPSVFLFPPKPKDTLMISRTPEVTCVVVDVSHEDPEVKFNWYVDGVEVHNAKTKPREEQYNSTYRVVSVLTVLHQDWLNGKEYKCKVSNKALPAPIEKTISKAKGQPREPQVYTLPPSREEMTKNQVSLTCLVKGFYPSDIAVEWESNGQPENNYKTTPPVLDSDGSFFLYSKLTVDKSRWQQGNVFSCSVMHEALHNHYTQKSLSLSPGK

SEQ ID NO: 43 - protein, 220 aa, artificial
  9E4 LC
DIQMTQSPSSLSASVGDRVTITCKSIQTLLYSSNQKNYLAWFQQKPGKAPKLLIYWASIRKSGVPSRFSGSGSGTDFTLTISSLQPEDLATYYCQQYYSYPLTFGGGTKLEIKRTVAAPSVFIFPPSDEQLKSGTASVVCLLNNFYPREAKVQWKVDNALQSGNSQESVTEQDSKDSTYSLSSTLTLSKADYEKHKVYACEVTHQGLSSPVTKSFNRGEC